European Patent Application EP 4 640 841 A1, published October 29, 2025. Title: Immuno Thermal Shift Assay. Applicant: Westfaelische Wilhelms-Universitaet Muenster. Application EP. The sequence listing filed with the application follows.

SEQUENCE LISTING (2 sequences)

SEQ ID NO: 1 - DNA, 40 bp, synthetic construct
  source 1..40: mol_type = other DNA
cattctggcgggatcccgggtgcagcccaccgaatccatc

SEQ ID NO: 2 - DNA, 43 bp, synthetic construct
  source 1..43: mol_type = other DNA
gctgcacccgggatccgaagttcacgcatttgttcttcacgag